European Patent Specification EP 3 787 702 B1, published August 7, 2024. Title: DERMAL FILLERS AND METHODS OF USE THEREOF. Applicant: SHOSEYOV, Oded ORR, Nadav SEROR MAKNOUZ, Jasmine ZARKA, Revital. The sequence listing filed with the application follows.

SEQUENCE LISTING (42 sequences)

SEQ ID NO: 1 - DNA, 4662 bp, Artificial Sequence
  Synthetic sequence containing the coding regions of the vacuolar signal sequence of barley gene for Thiol protease aleurain precursor fused to the human Collagen alpha 1(I) chain and flanking regions
gcgatgcatgtaatgtcatgagccacatgatccaatggccacaggaacgtaagaatgtagatagatttgattttgtccgttagatagcaaacaacattataaaaggtgtgtatcaatacgaactaattcactcattggattcatagaagtccattcctcctaagtatctaaaccatggctcacgctcgtgttctcctcctcgctctcgctgttttggcaacagctgctgtggctgtggcttctagttcttcttttgctgattcaaaccctattagacctgttactgatagagcagcttccactttggctcaattgcaagaggagggccaggttgagggccaagatgaggatatccctccaattacatgcgtgcaaaatggcttgcgttaccacgatagggatgtgtggaaacctgaaccttgtcgtatctgtgtgtgtgataacggcaaggtgctctgcgatgatgttatctgcgatgagacaaaaaattgccctggcgctgaagttcctgagggcgagtgttgccctgtgtgccctgatggttccgagtccccaactgatcaggaaactactggcgtggagggcccaaaaggagatactggtccacgtggtcctaggggtccagcaggtcctccaggtagagatggtattccaggccagcctggattgccaggaccaccaggcccacctggcccaccaggacctcctggtcttggtggaaatttcgctccacaactctcttatggctatgatgagaagtcaacaggtggtatttccgttccaggtcctatgggaccatccggaccaagaggtctcccaggtcctccaggtgctcctggacctcaaggctttcaaggacctccaggcgaaccaggagaaccaggcgcttctggaccaatgggcccaaggggaccacctggcccaccaggaaaaaatggcgatgatggcgaagctggaaagcctggtcgtcctggagagagaggtcctcctggcccacagggtgcaagaggcttgccaggaactgctggcttgcctggaatgaagggacataggggcttctccggcctcgatggcgctaagggtgatgctggccctgctggaccaaagggcgagccaggttcccctggagaaaacggtgctcctggacaaatgggtcctcgtggacttccaggagaaaggggtcgtccaggcgctccaggaccagcaggtgctaggggaaacgatggtgcaacaggcgctgctggccctcctggcccaactggtcctgctggccctccaggattcccaggcgcagttggagctaaaggagaagcaggaccacagggccctaggggttctgaaggacctcagggtgttagaggtgaaccaggtcctccaggcccagctggagcagctggtccagcaggaaatccaggtgctgatggtcaacctggagctaagggcgctaatggcgcaccaggtatcgcaggcgcaccaggttttcctggcgctagaggcccaagtggtcctcaaggaccaggtggaccaccaggtccaaaaggcaattctggcgaacctggcgctccaggttctaaaggagatactggtgctaaaggcgaaccaggacctgttggtgttcagggtcctcctggtcctgctggagaagaaggaaaaagaggtgctcgtggagaaccaggaccaactggacttcctggacctcctggtgaacgtggcggacctggctcaaggggtttccctggagctgatggagtggcaggtccaaaaggccctgctggagagagaggttcaccaggtccagctggtcctaagggctcccctggtgaagcaggtagaccaggcgaagcaggattgccaggcgcaaagggattgacaggctctcctggtagtcctggcccagatggaaaaacaggcccaccaggtccagcaggacaagatggacgtccaggcccaccaggtcctcctggagcaaggggacaagctggcgttatgggttttccaggacctaaaggtgctgctggagagccaggaaaggcaggtgaaagaggagttcctggtccaccaggagcagtgggtcctgctggcaaagatggtgaagctggagcacagggccctccaggccctgctggcccagctggcgaacgtggagaacaaggcccagctggtagtccaggatttcaaggattgcctggccctgctggccctccaggagaagcaggaaaacctggagaacaaggagttcctggtgatttgggagcacctggaccttcaggagcacgtggtgaaagaggcttccctggcgagaggggtgttcaaggtccaccaggtccagcaggacctagaggtgctaatggcgctcctggcaacgatggagcaaaaggtgatgctggtgctcctggcgcacctggaagtcagggtgctcctggattgcaaggaatgcctggagagaggggtgctgctggcttgccaggcccaaagggcgataggggtgatgctggaccaaaaggtgctgatggatccccaggaaaagatggagttcgtggtcttactggcccaatcggacctccaggccctgctggcgctccaggtgataagggcgaaagtggcccaagtggacctgctggacctactggtgctagaggtgcacctggtgataggggtgaacctggaccacctggtccagctggttttgctggtcctcctggagctgatggacaacctggcgcaaagggtgaaccaggtgatgctggcgcaaagggagatgctggtccacctggacctgctggtccagcaggcccccctgggccaatcggtaatgttggagcaccaggtgctaagggagctaggggttccgctggtccacctggagcaacaggatttccaggcgctgctggtagagttggcccaccaggcccatccggaaacgcaggccctcctggtcctccaggtcctgctggcaaggagggtggcaaaggaccaaggggcgaaactggccctgctggtagacctggcgaagttggccctcctggaccaccaggtccagcaggagaaaaaggttccccaggagctgatggcccagctggtgctccaggaactccaggccctcaaggtattgctggacagagaggcgttgtgggactccctggtcaaaggggagagagaggatttccaggcttgccaggacctagtggagaacctggaaaacaaggcccatcaggcgctagtggagagcgtggacctcctggccctatgggacctcctggattggctggcccacctggcgaatcaggtcgtgaaggcgcaccaggcgcagaaggatcacctggaagagatggatcccctggtgctaaaggcgatcgtggagaaactggtccagcaggcccaccaggcgcaccaggtgcacctggcgctccaggacctgtgggaccagctggaaaatccggagataggggcgagacaggcccagcaggaccagctggacctgttggccctgctggcgctcgtggaccagcaggacctcaaggaccaaggggagataagggagaaacaggcgaacaaggcgataggggcattaagggtcataggggttttagtggcctccagggtcctcctggcccacctggatcaccaggagaacagggaccatctggtgcttccggcccagctggtccaagaggacctccaggatcagctggtgcacctggaaaagatggtcttaacggtctcccaggaccaatcggccctccaggacctagaggaagaacaggagatgctggccctgttggccctccaggacctcctggtccaccaggtccacctggtcctccatcagctggattcgatttttcatttcttccacagccaccacaagagaaagctcacgatggcggcagatattaccgtgctgatgatgctaacgttgttagggatagagatttggaagtggatacaactttgaaatccctctcccagcaaattgaaaacattagatctccagaaggttcacgtaaaaacccagctagaacatgtcgtgatttgaaaatgtgtcactccgattggaaaagtggtgaatactggattgatccaaatcagggctgtaatctcgatgctatcaaagttttctgtaacatggaaacaggcgaaacatgcgtttatcctactcaaccttccgtggctcagaaaaattggtacatctcaaaaaatcctaaagataagaggcacgtttggttcggtgaaagtatgactgatggatttcaatttgagtacggcggtcaaggtagtgatccagctgatgtggctattcaactcacatttttgcgtcttatgtccacagaggcatcacaaaacatcacttaccactgcaaaaacagtgtggcttatatggatcaacaaacaggaaaccttaagaaggctcttcttttgaagggctcaaacgagattgagattagagcagagggcaactcaaggtttacttattcagttactgttgatggctgcacttcacatactggcgcttggggtaaaacagttatcgagtataagactacaaaaacatcaagactcccaatcattgatgttgctcctctcgatgttggcgctcctgatcaagagttcggttttgatgtgggcccagtttgtttcctctaatgagctcgcggccgcatc

SEQ ID NO: 2 - DNA, 4662 bp, Artificial Sequence; identical to SEQ ID NO: 1
  Synthetic sequence of the vacuolar signal sequence of barley gene for Thiol protease aleurain precursor fused to the human Collagen alpha 1(I) chain and flanking regions
  CDS (175)..(4644)

SEQ ID NO: 3 - protein, 1489 aa, Artificial Sequence
  Synthetic Construct
MAHARVLLLALAVLATAAVAVASSSSFADSNPIRPVTDRAASTLAQLQEEGQVEGQDEDIPPITCVQNGLRYHDRDVWKPEPCRICVCDNGKVLCDDVICDETKNCPGAEVPEGECCPVCPDGSESPTDQETTGVEGPKGDTGPRGPRGPAGPPGRDGIPGQPGLPGPPGPPGPPGPPGLGGNFAPQLSYGYDEKSTGGISVPGPMGPSGPRGLPGPPGAPGPQGFQGPPGEPGEPGASGPMGPRGPPGPPGKNGDDGEAGKPGRPGERGPPGPQGARGLPGTAGLPGMKGHRGFSGLDGAKGDAGPAGPKGEPGSPGENGAPGQMGPRGLPGERGRPGAPGPAGARGNDGATGAAGPPGPTGPAGPPGFPGAVGAKGEAGPQGPRGSEGPQGVRGEPGPPGPAGAAGPAGNPGADGQPGAKGANGAPGIAGAPGFPGARGPSGPQGPGGPPGPKGNSGEPGAPGSKGDTGAKGEPGPVGVQGPPGPAGEEGKRGARGEPGPTGLPGPPGERGGPGSRGFPGADGVAGPKGPAGERGSPGPAGPKGSPGEAGRPGEAGLPGAKGLTGSPGSPGPDGKTGPPGPAGQDGRPGPPGPPGARGQAGVMGFPGPKGAAGEPGKAGERGVPGPPGAVGPAGKDGEAGAQGPPGPAGPAGERGEQGPAGSPGFQGLPGPAGPPGEAGKPGEQGVPGDLGAPGPSGARGERGFPGERGVQGPPGPAGPRGANGAPGNDGAKGDAGAPGAPGSQGAPGLQGMPGERGAAGLPGPKGDRGDAGPKGADGSPGKDGVRGLTGPIGPPGPAGAPGDKGESGPSGPAGPTGARGAPGDRGEPGPPGPAGFAGPPGADGQPGAKGEPGDAGAKGDAGPPGPAGPAGPPGPIGNVGAPGAKGARGSAGPPGATGFPGAAGRVGPPGPSGNAGPPGPPGPAGKEGGKGPRGETGPAGRPGEVGPPGPPGPAGEKGSPGADGPAGAPGTPGPQGIAGQRGVVGLPGQRGERGFPGLPGPSGEPGKQGPSGASGERGPPGPMGPPGLAGPPGESGREGAPGAEGSPGRDGSPGAKGDRGETGPAGPPGAPGAPGAPGPVGPAGKSGDRGETGPAGPAGPVGPAGARGPAGPQGPRGDKGETGEQGDRGIKGHRGFSGLQGPPGPPGSPGEQGPSGASGPAGPRGPPGSAGAPGKDGLNGLPGPIGPPGPRGRTGDAGPVGPPGPPGPPGPPGPPSAGFDFSFLPQPPQEKAHDGGRYYRADDANVVRDRDLEVDTTLKSLSQQIENIRSPEGSRKNPARTCRDLKMCHSDWKSGEYWIDPNQGCNLDAIKVFCNMETGETCVYPTQPSVAQKNWYISKNPKDKRHVWFGESMTDGFQFEYGGQGSDPADVAIQLTFLRLMSTEASQNITYHCKNSVAYMDQQTGNLKKALLLKGSNEIEIRAEGNSRFTYSVTVDGCTSHTGAWGKTVIEYKTTKTSRLPIIDVAPLDVGAPDQEFGFDVGPVCFL

SEQ ID NO: 4 - DNA, 4362 bp, Artificial Sequence
  Synthetic sequence containing the coding regions of the vacuolar signal sequence of barley gene for Thiol protease aleurain precursor fused to the human Collagen alpha 2(I) chain and flanking regions
gcgatgcatgtaatgtcatgagccacatgatccaatggccacaggaacgtaagaatgtagatagatttgattttgtccgttagatagcaaacaacattataaaaggtgtgtatcaatacgaactaattcactcattggattcatagaagtccattcctcctaagtatctaaaccatggctcacgctcgtgttctcctcctcgctctcgctgttttggcaacagctgctgtggctgtggcttcaagttctagttttgctgattccaacccaattcgtccagttactgatagagcagcttccactttggctcaattgcttcaagaagaaactgtgaggaagggccctgctggcgataggggccctaggggcgaaaggggtccaccaggacctccaggcagggatggcgaagatggtccaactggccctcctggacctcctggccctccagggccacccggcttgggcggaaacttcgcagctcaatacgatggcaagggtgttggtcttggtcctggtcctatgggcttgatgggacctagaggcccacctggtgctgctggtgctcctggaccacagggttttcagggaccagctggcgagccaggagagccaggccaaacaggaccagctggtgcaaggggacctgctggacctcctggaaaagctggtgaagatggtcacccaggcaaaccaggacgtcctggcgaaagaggtgttgttggaccacaaggcgctaggggatttccaggtacacctggattgccaggttttaagggcattcgtggtcataacggcctcgatggattgaagggacagcctggcgcacctggcgttaagggtgaacctggagcaccaggtgaaaacggtactcctggccagactggtgcaagaggactcccaggtgaaaggggtagagttggtgctcctggacctgctggagctaggggtagtgatggtagtgttggtcctgtgggccctgctggtccaatcggttccgctggcccacctggattcccaggcgctccaggacctaaaggagaaatcggtgctgtgggtaacgcaggtcctactggtccagcaggtcctcgtggagaagtgggattgccaggactttctggtccagtgggccctccaggcaaccctggagctaacggcttgacaggagctaaaggcgcagcaggactccctggagtggctggcgcaccaggattgcctggtccaaggggtatcccaggccctgttggcgcagctggagctactggtgcacgtggacttgttggcgaaccaggccctgctggatcaaaaggcgagtctggaaataagggagaacctggttctgctggacctcaaggtcctcctggaccttctggagaagaaggaaaaaggggaccaaatggcgaggctggatcagcaggtccaccaggaccacctggacttcgtggatcccctggtagtagaggacttccaggcgctgatggtagagcaggcgttatgggaccaccaggaagtagaggagcatccggtccagcaggagttaggggtcctaacggagatgctggtagaccaggtgaaccaggtcttatgggcccaaggggcctcccaggtagtccaggaaatatcggccctgctggaaaagaaggccctgttggacttccaggtattgatggacgtcctggccctattggcccagcaggtgcaagaggagaacctggcaatattggatttccaggaccaaagggtccaacaggcgatcctggaaaaaatggagataagggtcatgctggattggcaggcgcaaggggcgctcctggtccagatggaaacaacggcgcacagggtccacctggccctcagggtgttcaaggcggaaaaggcgaacaaggcccagctggaccaccaggctttcaaggcttgccaggaccaagtggtccagcaggtgaagttggcaagccaggcgagcgtggacttcatggcgagtttggactccctggaccagcaggaccaaggggtgaaagaggccctcctggagagagtggcgctgctggaccaacaggcccaatcggtagtagaggtcctagtggacctccaggcccagatggaaataagggtgaaccaggagttgtgggcgctgttggaacagctggtccttcaggaccatcaggactcccaggcgagagaggcgctgctggcattcctggaggaaaaggtgaaaaaggcgaacctggcctccgtggcgaaatcggaaatcctggacgtgatggtgctcgtggtgcacacggcgctgtgggcgctccaggccctgctggtgctactggtgatagaggagaggctggcgcagctggcccagcaggtcctgctggcccaaggggtagtcctggtgaaagaggcgaagttggacctgctggccctaacggctttgctggccctgctggagcagcaggtcaacctggcgctaaaggtgaaaggggcggaaagggcccaaaaggtgaaaatggcgttgtgggaccaactggtccagtgggcgcagctggacctgctggtccaaatggaccaccaggaccagcaggtagtagaggagatggtggacctccaggaatgacaggttttccaggtgctgctggtagaacaggacctcctggtcctagtggtatttctggtccaccaggaccaccaggtcctgctggaaaagaaggattgaggggtccacgtggtgatcaaggaccagtgggcagaactggtgaagttggcgcagtgggaccacctggttttgctggagaaaagggcccttctggagaggcaggaacagctggtcctcctggtacacctggacctcaaggacttttgggtgcacctggtattctcggattgccaggaagtaggggcgaacgtggacttcctggcgtggcaggagcagttggagaacctggccctctcggaatcgcaggcccaccaggcgcaagaggaccaccaggagctgttggatcaccaggcgtgaatggtgcacctggcgaggctggtcgtgatggaaacccaggaaatgatggcccaccaggaagagatggtcaacctggacacaaaggcgagaggggctacccaggaaatattggcccagttggtgctgctggcgcaccaggcccacacggtccagttggaccagcaggaaaacacggtaatcgtggcgaaacaggcccttcaggcccagtgggacctgctggtgctgttggcccaagaggaccatctggacctcaaggcattagaggcgataagggagagcctggcgaaaaaggacctagaggcttgcctggttttaaaggacacaacggtctccaaggacttccaggtatcgctggtcatcatggagatcagggtgctcctggatcagtgggtccagcaggtcctagaggcccagcaggcccttccggtccagcaggaaaggatggacgtactggccaccctggaactgtgggccctgctggaattagaggtcctcaaggtcatcagggccctgctggccctccaggtccaccaggtcctccaggcccaccaggagtttcaggtggtggttacgattttggttacgatggtgatttttaccgtgctgatcaacctagaagtgctccttctctccgtcctaaagattatgaagttgatgctactttgaaatcacttaacaaccagattgagactcttctcacacctgagggatcaagaaagaatccagcacgtacatgccgtgatctcagacttagtcacccagagtggtcaagtggctattattggattgatcctaatcagggttgtacaatggaggctatcaaagtttactgtgattttccaactggagagacatgtattagggcacaacctgagaacattccagctaaaaattggtatcgttcctctaaagataagaaacatgtttggctcggagagactattaacgctggttctcagttcgagtataatgttgagggcgttacttctaaagagatggcaactcagctcgcttttatgagattgctcgctaactacgcatcccaaaacatcacttatcactgcaaaaattccattgcatatatggatgaggagacaggaaatttgaagaaagcagttattctccaaggtagtaacgatgttgagcttgtggctgagggaaatagtagattcacttacacagttttggtggatggatgctcaaagaaaactaatgagtggggcaagacaatcattgagtacaagacaaataagccttctaggctcccatttctcgatattgcacctcttgatatcggaggagctgatcacgagttttttgttgatatcggacctgtttgttttaagtaatgagctcgcggccgcatc

SEQ ID NO: 5 - DNA, 4362 bp, Artificial Sequence; identical to SEQ ID NO: 4
  Synthetic sequence of the vacuolar signal sequence of barley gene for Thiol protease aleurain precursor fused to the human Collagen alpha 2(I) chain and flanking regions
  CDS (175)..(4344)

SEQ ID NO: 6 - protein, 1389 aa, Artificial Sequence
  Synthetic Construct
MAHARVLLLALAVLATAAVAVASSSSFADSNPIRPVTDRAASTLAQLLQEETVRKGPAGDRGPRGERGPPGPPGRDGEDGPTGPPGPPGPPGPPGLGGNFAAQYDGKGVGLGPGPMGLMGPRGPPGAAGAPGPQGFQGPAGEPGEPGQTGPAGARGPAGPPGKAGEDGHPGKPGRPGERGVVGPQGARGFPGTPGLPGFKGIRGHNGLDGLKGQPGAPGVKGEPGAPGENGTPGQTGARGLPGERGRVGAPGPAGARGSDGSVGPVGPAGPIGSAGPPGFPGAPGPKGEIGAVGNAGPTGPAGPRGEVGLPGLSGPVGPPGNPGANGLTGAKGAAGLPGVAGAPGLPGPRGIPGPVGAAGATGARGLVGEPGPAGSKGESGNKGEPGSAGPQGPPGPSGEEGKRGPNGEAGSAGPPGPPGLRGSPGSRGLPGADGRAGVMGPPGSRGASGPAGVRGPNGDAGRPGEPGLMGPRGLPGSPGNIGPAGKEGPVGLPGIDGRPGPIGPAGARGEPGNIGFPGPKGPTGDPGKNGDKGHAGLAGARGAPGPDGNNGAQGPPGPQGVQGGKGEQGPAGPPGFQGLPGPSGPAGEVGKPGERGLHGEFGLPGPAGPRGERGPPGESGAAGPTGPIGSRGPSGPPGPDGNKGEPGVVGAVGTAGPSGPSGLPGERGAAGIPGGKGEKGEPGLRGEIGNPGRDGARGAHGAVGAPGPAGATGDRGEAGAAGPAGPAGPRGSPGERGEVGPAGPNGFAGPAGAAGQPGAKGERGGKGPKGENGVVGPTGPVGAAGPAGPNGPPGPAGSRGDGGPPGMTGFPGAAGRTGPPGPSGISGPPGPPGPAGKEGLRGPRGDQGPVGRTGEVGAVGPPGFAGEKGPSGEAGTAGPPGTPGPQGLLGAPGILGLPGSRGERGLPGVAGAVGEPGPLGIAGPPGARGPPGAVGSPGVNGAPGEAGRDGNPGNDGPPGRDGQPGHKGERGYPGNIGPVGAAGAPGPHGPVGPAGKHGNRGETGPSGPVGPAGAVGPRGPSGPQGIRGDKGEPGEKGPRGLPGFKGHNGLQGLPGIAGHHGDQGAPGSVGPAGPRGPAGPSGPAGKDGRTGHPGTVGPAGIRGPQGHQGPAGPPGPPGPPGPPGVSGGGYDFGYDGDFYRADQPRSAPSLRPKDYEVDATLKSLNNQIETLLTPEGSRKNPARTCRDLRLSHPEWSSGYYWIDPNQGCTMEAIKVYCDFPTGETCIRAQPENIPAKNWYRSSKDKKHVWLGETINAGSQFEYNVEGVTSKEMATQLAFMRLLANYASQNITYHCKNSIAYMDEETGNLKKAVILQGSNDVELVAEGNSRFTYTVLVDGCSKKTNEWGKTIIEYKTNKPSRLPFLDIAPLDIGGADHEFFVDIGPVCFK

SEQ ID NO: 7 - DNA, 127 bp, Artificial Sequence
  Synthetic sequence containing the coding region of the appoplast signal of Arabidopsis thaliana endo-1,4-beta-glucanase and flanking regions
gccatggctaggaagtctttgattttcccagtgattcttcttgctgtgcttcttttctctccacctatttactctgctggacacgattatagggatgctcttaggaagtcatctatggctcaattgc

SEQ ID NO: 8 - DNA, 127 bp, Artificial Sequence; identical to SEQ ID NO: 7
  Synthetic sequence of the appoplast signal of Arabidopsis thaliana endo-1,4-beta-glucanase and flanking regions
  CDS (10)..(120)

SEQ ID NO: 9 - protein, 37 aa, Artificial Sequence
  Synthetic Construct
RKSLIFPVILLAVLLFSPPIYSAGHDYRDALRKSSMA

SEQ ID NO: 10 - DNA, 1037 bp, Artificial Sequence
  Chrysanthemum rbcS1 promoter and 5' UTR
aaatggcgcgccaagcttagacaaacaccccttgttatacaaagaatttcgctttacaaaatcaaattcgagaaaataatatatgcactaaataagatcattcggatccaatctaaccaattacgatacgctttgggtacacttgatttttgtttcagtagttacatatatcttgttttatatgctatctttaaggatcttcactcaaagactatttgttgatgttcttgatggggctcggaagatttgatatgatacactctaatctttaggagataccagccaggattatattcagtaagacaatcaaattttacgtgttcaaactcgttatcttttcatttaatggatgagccagaatctctatagaatgattgcaatcgagaatatgttcggccgatatccctttgttggcttcaatattctacatatcacacaagaatcgaccgtattgtaccctctttccataaaggaacacacagtatgcagatgcttttttcccacatgcagtaacataggtattcaaaaatggctaaaagaagttggataacaaattgacaactatttccatttctgttatataaatttcacaacacacaaaagcccgtaatcaagagtctgcccatgtacgaaataacttctattatttggtattgggcctaagcccagctcagagtacgtgggggtaccacatataggaaggtaacaaaatactgcaagatagccccataacgtaccagcctctccttaccacgaagagataagatataagacccaccctgccacgtgtcacatcgtcatggtggttaatgataagggattacatccttctatgtttgtggacatgatgcatgtaatgtcatgagccacatgatccaatggccacaggaacgtaagaatgtagatagatttgattttgtccgttagatagcaaacaacattataaaaggtgtgtatcaatacgaactaattcactcattggattcatagaagtccattcctcctaagtatctaaacatatgcaattgtcgactaaa

SEQ ID NO: 11 - DNA, 975 bp, Artificial Sequence
  Chrysanthemum rbcS1  3'UTR and terminator
aaaaggatccgcggccgcataagttttactatttaccaagacttttgaatattaaccttcttgtaacgagtcggttaaatttgattgtttagggttttgtattatttttttttggtcttttaattcatcactttaattccctaattgtctgttcatttcgttgtttgtttccggatcgataatgaaatgtaagagatatcatatataaataataaattgtcgtttcatatttgcaatctttttttacaaacctttaattaattgtatgtatgacattttcttcttgttatattagggggaaataatgttaaataaaagtacaaaataaactacagtacatcgtactgaataaattacctagccaaaaagtacacctttccatatacttcctacatgaaggcattttcaacattttcaaataaggaatgctacaaccgcataataacatccacaaatttttttataaaataacatgtcagacagtgattgaaagattttattatagtttcgttatcttcttttctcattaagcgaatcactacctaacacgtcattttgtgaaatattttttgaatgtttttatatagttgtagcattcctcttttcaaattagggtttgtttgagatagcatttcagccggttcatacaacttaaaagcatactctaatgctggaaaaaagactaaaaaatcttgtaagttagcgcagaatattgacccaaattatatacacacatgaccccatatagagactaattacacttttaaccactaataattattactgtattataacatctactaattaaacttgtgagtttttgctagaattattatcatatatactaaaaggcaggaacgcaaacattgccccggtactgtagcaactacggtagacgcattaattgtctatagtggacgcattaattaaccaaaaccgcctctttccccttcttcttgaagcttgagctctttt

SEQ ID NO: 12 - DNA, 1633 bp, Artificial Sequence
  Synthetic sequence containing the coding regions of the vacuolar signal sequence of barley gene for Thiol protease aleurain precursor fused to the human Prolyl 4-hydroxylase beta subunit and flanking regions
ctcgagtaaaccatggctcatgctagggttttgcttttggctcttgctgttcttgctactgctgctgttgctgtggcttcttcttcatctttcgctgattctaacccaattaggccagtgactgatagagctgcttctactcttgctcaattggtcgacatggatgctccagaagaggaggatcacgttcttgtgcttaggaagtctaacttcgctgaagctcttgctgctcacaagtaccttcttgtggagttttatgctccttggtgcggacattgcaaagctcttgctccagagtatgctaaggctgctggaaagttgaaggctgagggatctgaaattaggcttgctaaagtggatgctactgaggagtctgatcttgctcaacagtacggagttaggggatacccaactattaagttcttcaggaacggagatactgcttctccaaaggagtatactgctggaagggaggctgatgatattgtgaactggcttaagaagagaactggaccagctgctactactcttccagatggagctgctgctgaatctcttgtggagtcatctgaggtggcagtgattggattcttcaaggatgtggagtctgattctgctaagcagttccttcaagctgctgaggctattgatgatattccattcggaattacttctaactctgatgtgttctctaagtaccagcttgataaggatggagtggtgcttttcaagaaattcgatgagggaaggaacaatttcgagggagaggtgacaaaggagaaccttcttgatttcattaagcacaaccagcttccacttgtgattgagttcactgagcagactgctccaaagattttcggaggagagattaagactcacattcttcttttccttccaaagtctgtgtctgattacgatggaaagttgtctaacttcaagactgctgctgagtctttcaagggaaagattcttttcattttcattgattctgatcacactgataaccagaggattcttgagttcttcggacttaagaaggaagagtgcccagctgttaggcttattactcttgaggaggagatgactaagtacaagccagagtctgaagaacttactgctgagaggattactgagttctgccacagattccttgagggaaagattaagccacaccttatgtctcaagagcttccagaggattgggataagcagccagttaaggtgttggtgggtaaaaacttcgaggatgtggctttcgatgagaagaagaacgtgttcgtggagttctacgcaccttggtgtggtcactgtaagcagcttgctccaatttgggataagttgggagagacttacaaggatcacgagaacattgtgattgctaagatggattctactgctaacgaggtggaggctgttaaggttcactctttcccaactttgaagttcttcccagcttctgctgataggactgtgattgattacaacggagaaaggactcttgatggattcaagaagttccttgagtctggaggacaagatggagctggagatgatgatgatcttgaggatttggaagaagctgaggagccagatatggaggaggatgatgatcagaaggctgtgtgatgagctc

SEQ ID NO: 13 - protein, 537 aa, Artificial Sequence
  Synthetic sequence containing the vacuolar signal sequence of barley gene for Thiol protease aleurain precursor fused to the human Prolyl 4-hydroxylase beta subunit and flanking regions
MAHARVLLLALAVLATAAVAVASSSSFADSNPIRPVTDRAASTLAQLVDMDAPEEEDHVLVLRKSNFAEALAAHKYLLVEFYAPWCGHCKALAPEYAKAAGKLKAEGSEIRLAKVDATEESDLAQQYGVRGYPTIKFFRNGDTASPKEYTAGREADDIVNWLKKRTGPAATTLPDGAAAESLVESSEVAVIGFFKDVESDSAKQFLQAAEAIDDIPFGITSNSDVFSKYQLDKDGVVLFKKFDEGRNNFEGEVTKENLLDFIKHNQLPLVIEFTEQTAPKIFGGEIKTHILLFLPKSVSDYDGKLSNFKTAAESFKGKILFIFIDSDHTDNQRILEFFGLKKEECPAVRLITLEEEMTKYKPESEELTAERITEFCHRFLEGKIKPHLMSQELPEDWDKQPVKVLVGKNFEDVAFDEKKNVFVEFYAPWCGHCKQLAPIWDKLGETYKDHENIVIAKMDSTANEVEAVKVHSFPTLKFFPASADRTVIDYNGERTLDGFKKFLESGGQDGAGDDDDLEDLEEAEEPDMEEDDDQKAV

SEQ ID NO: 14 - DNA, 1723 bp, Artificial Sequence
  Synthetic sequence containing the coding regions of the vacuolar signal sequence of barley gene for Thiol protease aleurain precursor fused to the human Prolyl 4-hydroxylase alpha-1 subunit and flanking regions
ctcgagtaaaccatggctcatgctagggttttgcttttggctcttgctgttcttgctactgctgctgttgctgtggcttcttcttcatctttcgctgattctaacccaattaggccagtgactgatagagctgcttctactcttgctcaattggtcgacatgcacccaggattcttcacttctattggacagatgactgatcttattcacactgagaaggatcttgtgacttctcttaaggattacattaaggctgaggaggataagttggagcagattaagaagtgggctgagaagttggataggcttacttctactgctacaaaagatccagagggattcgttggtcatccagtgaacgctttcaagttgatgaagaggcttaacactgagtggagtgagcttgagaaccttgtgcttaaggatatgtctgatggattcatttctaaccttactattcagaggcagtacttcccaaatgatgaggatcaagtgggagctgctaaggctcttcttaggcttcaggatacttacaaccttgatactgatacaatttctaagggaaaccttccaggagttaagcacaagtctttccttactgctgaggattgcttcgagcttggaaaggttgcatacactgaggctgattactaccacactgagctttggatggaacaagctcttaggcaacttgatgagggagagatttctactattgataaggtgtcagtgcttgattacctttcttacgctgtgtaccagcagggtgatcttgataaggctcttttgcttactaagaagttgcttgagcttgatccagaacatcagagggctaacggaaaccttaagtacttcgagtacattatggctaaggaaaaggatgtgaacaagtctgcttctgatgatcagtctgatcaaaagactactccaaagaagaagggagtggctgttgattatcttcctgagaggcagaagtatgagatgttgtgtaggggagagggtattaagatgactccaaggaggcagaagaagttgttctgcaggtatcacgatggaaacaggaacccaaagttcattcttgctccagctaagcaagaagatgagtgggataagccaaggattattaggttccacgatattatttctgatgctgagattgagattgtgaaggatcttgctaagccaagacttaggagggctactatttctaaccctattactggtgatcttgagactgtgcactacaggatttctaagtctgcttggctttctggatacgagaacccagtggtgtctaggattaacatgaggattcaggatcttactggacttgatgtgtctactgctgaggagcttcaagttgctaactacggagttggaggacaatatgagccacacttcgatttcgctaggaaggatgagccagatgcttttaaggagcttggaactggaaacaggattgctacttggcttttctacatgtctgatgtttctgctggaggagctactgttttcccagaagtgggagcttctgtttggccaaagaagggaactgctgtgttctggtacaaccttttcgcttctggagagggagattactctactaggcatgctgcttgcccagttcttgttggaaacaagtgggtgtcaaacaagtggcttcatgagaggggacaagagtttagaaggccatgcactctttctgagcttgagtgatgagctc

SEQ ID NO: 15 - protein, 567 aa, Artificial Sequence
  Synthetic sequence containing the vacuolar signal sequence of barley gene for Thiol protease aleurain precursor fused to the human Prolyl 4-hydroxylase alpha-1 subunit and flanking regions
MAHARVLLLALAVLATAAVAVASSSSFADSNPIRPVTDRAASTLAQLVDMHPGFFTSIGQMTDLIHTEKDLVTSLKDYIKAEEDKLEQIKKWAEKLDRLTSTATKDPEGFVGHPVNAFKLMKRLNTEWSELENLVLKDMSDGFISNLTIQRQYFPNDEDQVGAAKALLRLQDTYNLDTDTISKGNLPGVKHKSFLTAEDCFELGKVAYTEADYYHTELWMEQALRQLDEGEISTIDKVSVLDYLSYAVYQQGDLDKALLLTKKLLELDPEHQRANGNLKYFEYIMAKEKDVNKSASDDQSDQKTTPKKKGVAVDYLPERQKYEMLCRGEGIKMTPRRQKKLFCRYHDGNRNPKFILAPAKQEDEWDKPRIIRFHDIISDAEIEIVKDLAKPRLRRATISNPITGDLETVHYRISKSAWLSGYENPVVSRINMRIQDLTGLDVSTAEELQVANYGVGGQYEPHFDFARKDEPDAFKELGTGNRIATWLFYMSDVSAGGATVFPEVGASVWPKKGTAVFWYNLFASGEGDYSTRHAACPVLVGNKWVSNKWLHERGQEFRRPCTLSELE

SEQ ID NO: 16 - DNA, 928 bp, Artificial Sequence
  Synthetic sequence containing the coding regions of the vacuolar signal sequence of barley gene for Thiol protease aleurain precursor fused to the plant Prolyl 4-hydroxylase Plant and flanking regions
ctcgagtaaaccatggctcatgctagggttttgcttttggctcttgctgttcttgctactgctgctgttgctgtggcttcttcttcatctttcgctgattctaacccaattaggccagtgactgatagagctgcttctactcttgctcaattggtcgacatgcttggtattctttctcttccaaacgctaacaggaactcttctaagactaacgatcttactaacattgtgaggaagtctgagacttcttctggagatgaggagggaaatggagaaagatgggtggaagtgatttcttgggagccaagggctgttgtttaccacaacttccttactaatgaggagtgcgagcaccttatttctcttgctaagccatctatggtgaagtctactgtggtggatgagaaaactggaggatctaaggattcaagagtgaggacttcatctggtactttccttaggaggggacatgatgaagttgtggaagttattgagaagaggatttctgatttcactttcattccagtggagaacggagaaggacttcaagttcttcactaccaagtgggacaaaagtacgagccacactacgattacttccttgatgagttcaacactaagaacggaggacagaggattgctactgtgcttatgtacctttctgatgtggatgatggaggagagactgtttttccagctgctaggggaaacatttctgctgttccttggtggaacgagctttctaagtgtggaaaggagggactttctgtgcttccaaagaaaagggatgctcttcttttctggaacatgaggccagatgcttctcttgatccatcttctcttcatggaggatgcccagttgttaagggaaacaagtggtcatctactaagtggttccacgtgcacgagttcaaggtgtaatgagctc

SEQ ID NO: 17 - protein, 302 aa, Artificial Sequence
  Synthetic sequence containing the vacuolar signal sequence of barley gene for Thiol protease aleurain precursor fused to the plant Prolyl 4-hydroxylase Plant and flanking regions
MAHARVLLLALAVLATAAVAVASSSSFADSNPIRPVTDRAASTLAQLVDMLGILSLPNANRNSSKTNDLTNIVRKSETSSGDEEGNGERWVEVISWEPRAVVYHNFLTNEECEHLISLAKPSMVKSTVVDEKTGGSKDSRVRTSSGTFLRRGHDEVVEVIEKRISDFTFIPVENGEGLQVLHYQVGQKYEPHYDYFLDEFNTKNGGQRIATVLMYLSDVDDGGETVFPAARGNISAVPWWNELSKCGKEGLSVLPKKRDALLFWNMRPDASLDPSSLHGGCPVVKGNKWSSTKWFHVHEFKV

SEQ ID NO: 18 - DNA, 2689 bp, Artificial Sequence
  Synthetic sequence containing the coding regions of the human Procollagen C-proteinase and flanking regions
agatctatcgatgcatgccatggtaccgcgccatggctcaattggctgcaacatcaaggcctgaaagagtttggccagatggtgttattcctttcgttattggtggaaactttactggatctcagagagcagtttttagacaagctatgagacattgggaaaagcacacttgtgtgacattccttgaaaggactgatgaagattcttatattgtgttcacataccgtccatgtggatgctgctcatatgttggtagaaggggaggaggtccacaagcaatttctattggaaaaaactgcgataagttcggaattgtggtgcatgaattgggacatgttgttggtttctggcacgaacacacaaggccagatagggataggcacgtgtctattgtgagggaaaacattcagccaggtcaagagtacaattttcttaagatggaacctcaagaggtggaatctctcggagagacttacgacttcgactccatcatgcactacgcaaggaatactttcagcaggggcatcttcttggataccattgtgcctaagtacgaggtgaacggcgttaagccacctattggtcaaaggactaggctctctaagggtgatattgcacaggctaggaagctctacaaatgtccagcatgcggagaaactcttcaggattccactggcaacttctcatctccagagtacccaaacggatactctgctcatatgcactgtgtttggaggatctcagtgactcctggagagaagatcatcctcaacttcacttccctcgatctctatcgttctaggctctgttggtacgactatgtggaagtgagagatggcttctggagaaaggctccacttagaggaaggttctgcggatctaaacttcctgagccaatcgtgtctactgattccagattgtgggtggagttcaggtcctcttctaattgggttggcaagggcttttttgctgtgtacgaggctatttgtggcggcgacgtgaaaaaggactacggacatattcaaagtccaaattacccagatgattaccgtccttcaaaagtgtgtatttggaggattcaagtgagtgagggtttccatgttggattgacattccaatctttcgaaattgagagacacgattcatgcgcatacgattatttggaagtgagagatggacactctgaatcttctacacttattggaaggtactgcggttatgagaaacctgatgatattaagtctacttctagtaggttgtggcttaaatttgtgtcagatggttctattaacaaggctggtttcgcagtgaacttcttcaaggaagtggatgaatgctcaagacctaacagaggaggatgtgagcaaagatgccttaacactttgggaagttacaagtgttcttgcgatcctggatacgagttggctcctgataagagaagatgcgaagctgcttgcggtggttttttgacaaaattgaacggatctattacttctcctggatggccaaaagagtacccacctaataagaattgcatttggcagcttgttgcacctactcagtaccgtatttcattgcaattcgattttttcgagactgagggtaatgatgtgtgcaagtacgatttcgtggaagtgagatcaggtcttactgctgatagtaaattgcacggaaagttctgcggatctgaaaaaccagaagtgattacatcacagtacaacaatatgagggtggagttcaaatctgataatactgtttctaaaaaaggttttaaggcacatttcttttctgataaggacgagtgctctaaagataatggtggttgccagcaggattgcgtgaacacattcggttcatatgagtgccaatgccgtagtggatttgttcttcacgataacaaacatgattgcaaagaggcaggttgcgatcacaaggtgacatctacttcaggtactatcacatctccaaactggcctgataagtatccttcaaaaaaagaatgtacatgggcaatttcttctacaccaggtcatagggttaagttgacattcatggagatggatattgagagtcaaccagagtgcgcttatgatcatcttgaggtgttcgatggaagggatgctaaggctcctgttcttggtagattctgtggtagtaaaaagccagaaccagtgcttgcaacaggatctaggatgttccttagattctactctgataactcagttcagaggaaaggattccaagctagtcacgcaactgaatgcggtggacaagttagagcagatgttaagactaaggatctttactcacacgcacagttcggagataacaactaccctggaggagttgattgcgagtgggttattgtggctgaagagggatacggagttgagcttgttttccagacattcgaggtggaggaggaaactgattgcggttacgattatatggaactttttgatggatacgatagtactgctccaagacttggaaggtattgtggtagtggtccaccagaagaggtgtactcagctggagatagtgttcttgttaagttccacagtgatgatacaattactaagaagggattccatcttagatatacttcaactaagtttcaggatactcttcattctaggaagtaatgagctcgcggccgcatccaagcttctgcagacgcgtcgacgtc

SEQ ID NO: 19 - protein, 870 aa, Artificial Sequence
  Synthetic sequence containing the human Procollagen C-proteinase and flanking regions
MAQLAATSRPERVWPDGVIPFVIGGNFTGSQRAVFRQAMRHWEKHTCVTFLERTDEDSYIVFTYRPCGCCSYVGRRGGGPQAISIGKNCDKFGIVVHELGHVVGFWHEHTRPDRDRHVSIVRENIQPGQEYNFLKMEPQEVESLGETYDFDSIMHYARNTFSRGIFLDTIVPKYEVNGVKPPIGQRTRLSKGDIAQARKLYKCPACGETLQDSTGNFSSPEYPNGYSAHMHCVWRISVTPGEKIILNFTSLDLYRSRLCWYDYVEVRDGFWRKAPLRGRFCGSKLPEPIVSTDSRLWVEFRSSSNWVGKGFFAVYEAICGGDVKKDYGHIQSPNYPDDYRPSKVCIWRIQVSEGFHVGLTFQSFEIERHDSCAYDYLEVRDGHSESSTLIGRYCGYEKPDDIKSTSSRLWLKFVSDGSINKAGFAVNFFKEVDECSRPNRGGCEQRCLNTLGSYKCSCDPGYELAPDKRRCEAACGGFLTKLNGSITSPGWPKEYPPNKNCIWQLVAPTQYRISLQFDFFETEGNDVCKYDFVEVRSGLTADSKLHGKFCGSEKPEVITSQYNNMRVEFKSDNTVSKKGFKAHFFSDKDECSKDNGGCQQDCVNTFGSYECQCRSGFVLHDNKHDCKEAGCDHKVTSTSGTITSPNWPDKYPSKKECTWAISSTPGHRVKLTFMEMDIESQPECAYDHLEVFDGRDAKAPVLGRFCGSKKPEPVLATGSRMFLRFYSDNSVQRKGFQASHATECGGQVRADVKTKDLYSHAQFGDNNYPGGVDCEWVIVAEEGYGVELVFQTFEVEEETDCGYDYMELFDGYDSTAPRLGRYCGSGPPEEVYSAGDSVLVKFHSDDTITKKGFHLRYTSTKFQDTLHSRK

SEQ ID NO: 20 - DNA, 2912 bp, Artificial Sequence
  Synthetic sequence containing the coding regions of the human Procollagen I N-proteinase and flanking regions
gcgccatggctcaattgaggagaagggctaggagacacgcagctgatgatgattacaacattgaagttttgcttggtgttgatgatagtgtggtgcaattccacggaaaagagcatgttcagaaatatcttttgacacttatgaatattgtgaacgaaatctaccatgatgagtctttgggagcacacattaacgtggttcttgtgaggattattcttctttcatacggtaaatctatgtcacttattgagattggaaacccttctcagtctcttgagaatgtgtgcagatgggcataccttcaacagaagcctgatactggacacgatgagtatcacgatcacgctattttccttacaaggcaggatttcggtccaagtggaatgcaaggatatgctcctgttactggtatgtgccaccctgttaggtcttgtacacttaaccacgaggatggtttttcatctgctttcgtggtggctcatgagacaggtcatgttttgggaatggaacatgatggacagggtaatagatgtggagatgaagtgagacttggttcaattatggctcctcttgttcaagctgcttttcataggttccactggagtaggtgttcacagcaagagttgagtagataccttcattcttacgattgcttgcttgatgatccatttgctcatgattggccagctttgcctcaacttcctggattgcactactctatgaacgagcagtgcagatttgatttcggtcttggttacatgatgtgcacagctttcaggactttcgatccatgcaaacagttgtggtgttcacacccagataacccatatttctgtaaaacaaaaaaaggtccaccacttgatggtactatgtgcgcacctggaaagcactgcttcaagggacactgcatttggcttactcctgatattcttaaaagggatggatcatggggagcttggtctccattcggaagttgctcaagaacttgcggaacaggtgttaagtttagaactaggcagtgcgataatccacaccctgctaatggtggtagaacttgctctggacttgcttacgattttcagttgtgttctaggcaagattgccctgatagtcttgctgattttagagaagagcaatgtagacagtgggatctttactttgagcacggcgacgctcagcaccactggcttccacacgagcatagagatgcaaaagaaaggtgtcacctttattgcgagagtagagagactggagaggtggtgtcaatgaagagaatggtgcacgatggtacaaggtgttcttataaggatgcattctctttgtgtgtgaggggagattgcaggaaagtgggttgtgatggagtgattggatctagtaagcaagaagataagtgcggagtgtgcggaggagataactctcattgcaaggttgtgaaaggaacttttacaagatcaccaaaaaaacacggttacattaagatgttcgaaattcctgctggagcaaggcatttgcttattcaggaagtggatgcaacatctcaccacttggcagtgaaaaaccttgagactggaaaattcattttgaacgaggagaacgatgttgatgcatctagtaagactttcattgcaatgggtgttgaatgggagtatagggatgaggatggaagggaaacacttcaaacaatgggtcctcttcatggaacaattactgtgttggtgattccagtgggagatacaagggtgtcattgacatacaagtatatgattcacgaggatagtcttaacgttgatgataacaacgttttggaagaagattctgtggtttacgagtgggctcttaagaaatggtcaccttgctctaagccatgtggtggaggaagtcagttcactaagtatggttgtaggaggaggcttgatcataagatggttcataggggattttgcgcagcacttagtaagccaaaggcaattaggagggcttgtaaccctcaagaatgctcacaaccagtttgggtgacaggagagtgggagccatgttcacaaacatgcggaagaactggaatgcaagttagatcagttagatgcattcaacctcttcatgataacactacaagaagtgtgcacgcaaaacactgtaacgatgctaggccagagagtagaagagcttgctctagggaactttgccctggtagatggagggcaggaccttggagtcagtgctctgtgacatgtggaaacggtactcaggaaagacctgttccatgtagaactgctgatgatagtttcggaatttgtcaggaggaaaggccagaaacagctaggacttgtagacttggaccttgtcctaggaatatttctgatcctagtaaaaaatcatacgtggtgcaatggttgagtaggccagatccagattcaccaattaggaagatttcttcaaaaggacactgccagggtgataagagtattttctgcagaatggaagttcttagtaggtactgttctattccaggttataacaaactttcttgtaagagttgcaacttgtataacaatcttactaacgtggagggtagaattgaacctccaccaggaaagcacaacgatattgatgtgtttatgcctactcttcctgtgccaacagttgcaatggaagttagaccttctccatctactccacttgaggtgccacttaatgcatcaagtactaacgctactgaggatcacccagagactaacgcagttgatgagccttataagattcacggacttgaggatgaggttcagccaccaaaccttattcctaggaggccaagtccttacgaaaaaactagaaatcagaggattcaggagcttattgatgagatgaggaaaaaggagatgcttggaaagttctaatgagctcgcggccgcatc

SEQ ID NO: 21 - protein, 962 aa, Artificial Sequence
  Synthetic sequence containing the human Procollagen I N-proteinase and flanking regions
MAQLRRRARRHAADDDYNIEVLLGVDDSVVQFHGKEHVQKYLLTLMNIVNEIYHDESLGAHINVVLVRIILLSYGKSMSLIEIGNPSQSLENVCRWAYLQQKPDTGHDEYHDHAIFLTRQDFGPSGMQGYAPVTGMCHPVRSCTLNHEDGFSSAFVVAHETGHVLGMEHDGQGNRCGDEVRLGSIMAPLVQAAFHRFHWSRCSQQELSRYLHSYDCLLDDPFAHDWPALPQLPGLHYSMNEQCRFDFGLGYMMCTAFRTFDPCKQLWCSHPDNPYFCKTKKGPPLDGTMCAPGKHCFKGHCIWLTPDILKRDGSWGAWSPFGSCSRTCGTGVKFRTRQCDNPHPANGGRTCSGLAYDFQLCSRQDCPDSLADFREEQCRQWDLYFEHGDAQHHWLPHEHRDAKERCHLYCESRETGEVVSMKRMVHDGTRCSYKDAFSLCVRGDCRKVGCDGVIGSSKQEDKCGVCGGDNSHCKVVKGTFTRSPKKHGYIKMFEIPAGARHLLIQEVDATSHHLAVKNLETGKFILNEENDVDASSKTFIAMGVEWEYRDEDGRETLQTMGPLHGTITVLVIPVGDTRVSLTYKYMIHEDSLNVDDNNVLEEDSVVYEWALKKWSPCSKPCGGGSQFTKYGCRRRLDHKMVHRGFCAALSKPKAIRRACNPQECSQPVWVTGEWEPCSQTCGRTGMQVRSVRCIQPLHDNTTRSVHAKHCNDARPESRRACSRELCPGRWRAGPWSQCSVTCGNGTQERPVPCRTADDSFGICQEERPETARTCRLGPCPRNISDPSKKSYVVQWLSRPDPDSPIRKISSKGHCQGDKSIFCRMEVLSRYCSIPGYNKLSCKSCNLYNNLTNVEGRIEPPPGKHNDIDVFMPTLPVPTVAMEVRPSPSTPLEVPLNASSTNATEDHPETNAVDEPYKIHGLEDEVQPPNLIPRRPSPYEKTRNQRIQELIDEMRKKEMLGKF

SEQ ID NO: 22 - DNA, 2888 bp, Artificial Sequence
  Synthetic sequence containing the coding regions of the vacuolar signal sequence of barley gene for Thiol protease aleurain precursor fused to the human Lysyl hydroxylase 3 and flanking regions
gcgaattcgctagctatcactgaaaagacagcaagacaatggtgtctcgatgcaccagaaccacatctttgcagcagatgtgaagcagccagagtggtccacaagacgcactcagaaaaggcatcttctaccgacacagaaaaagacaaccacagctcatcatccaacatgtagactgtcgttatgcgtcggctgaagataagactgaccccaggccagcactaaagaagaaataatgcaagtggtcctagctccactttagctttaataattatgtttcattattattctctgcttttgctctctatataaagagcttgtattttcatttgaaggcagaggcgaacacacacacagaacctccctgcttacaaaccagatcttaaaccatggctcacgctagggttttgcttcttgctcttgctgttcttgctactgctgctgttgctgtggcttcttcaagttctttcgctgattctaacccaattaggccagtgactgatagagctgcttctactcttgctcaattgagatctatgtctgatagaccaaggggaagggatccagttaatccagagaagttgcttgtgattactgtggctactgctgagactgaaggataccttagattccttaggagtgctgagttcttcaactacactgtgaggactcttggacttggagaagaatggaggggaggagatgttgctagaactgttggaggaggacagaaagtgagatggcttaagaaagagatggagaagtacgctgatagggaggatatgattattatgttcgtggattcttacgatgtgattcttgctggatctccaactgagcttttgaagaaattcgttcagtctggatctaggcttcttttctctgctgagtctttttgttggccagaatggggacttgctgagcaatatccagaagtgggaactggaaagagattccttaactctggaggattcattggattcgctactactattcaccagattgtgaggcagtggaagtacaaggatgacgatgatgatcagcttttctacactaggctttaccttgatccaggacttagggagaagttgtctcttaaccttgatcacaagtctaggattttccagaaccttaacggtgctcttgatgaggttgtgcttaagttcgataggaacagagtgaggattaggaacgtggcttacgatactcttcctattgtggtgcatggaaacggaccaacaaaactccagcttaactaccttggaaactacgttccaaacggatggactccagaaggaggatgtggattctgcaatcaggataggagaactcttccaggaggacaaccaccaccaagagttttccttgctgtgttcgttgaacagccaactccattccttccaagattccttcagaggcttcttcttttggattacccaccagatagggtgacacttttccttcacaacaacgaggttttccacgagccacacattgctgattcttggccacagcttcaggatcatttctctgctgtgaagttggttggtccagaagaagctctttctccaggagaagctagggatatggctatggatttgtgcaggcaggatccagagtgcgagttctacttctctcttgatgctgatgctgtgcttactaaccttcagactcttaggattcttattgaggagaacaggaaagtgattgctccaatgctttctaggcacggaaagttgtggtctaatttctggggtgctctttctcctgatgagtactacgctagatcagaggactacgtggagcttgttcagagaaagagagtgggagtttggaacgttccttatatttctcaggcttacgtgattaggggagatactcttaggatggagcttccacagagggatgttttctctggatctgatactgatccagatatggctttctgcaagtctttcagggataagggaattttccttcacctttctaaccagcatgagttcggaagattgcttgctacttcaagatacgatactgagcaccttcatcctgatctttggcagattttcgataacccagtggattggaaggagcagtacattcacgagaactactctagggctcttgaaggagaaggaattgtggagcaaccatgcccagatgtttactggttcccacttctttctgagcaaatgtgcgatgagcttgttgctgagatggagcattacggacaatggagtggaggtagacatgaggattctaggcttgctggaggatacgagaacgttccaactgtggatattcacatgaagcaagtgggatacgaggatcaatggcttcagcttcttaggacttatgtgggaccaatgactgagtctcttttcccaggataccacactaaggctagggctgttatgaacttcgttgtgaggtatcgtccagatgagcaaccatctcttaggccacaccacgattcttctactttcactcttaacgtggctcttaaccacaagggacttgattatgagggaggaggatgccgtttccttagatacgattgcgtgatttcttcaccaagaaagggatgggctcttcttcatccaggaaggcttactcattaccacgagggacttccaactacttggggaactagatatattatggtgtctttcgtggatccatgactgctttaatgagatatgcgagacgcctatgatcgcatgatatttgctttcaattctgttgtgcacgttgtaaaaaacctgagcatgtgtagctcagatccttaccgccggtttcggttcattctaatgaatatatcacccgttactatcgtatttttatgaataatattctccgttcaatttactgattgtccagaattcgcg

SEQ ID NO: 23 - protein, 764 aa, Artificial Sequence
  Synthetic sequence containing the vacuolar signal sequence of barley gene for Thiol protease aleurain precursor fused to the human Lysyl hydroxylase 3 and flanking regions
MAHARVLLLALAVLATAAVAVASSSSFADSNPIRPVTDRAASTLAQLRSMSDRPRGRDPVNPEKLLVITVATAETEGYLRFLRSAEFFNYTVRTLGLGEEWRGGDVARTVGGGQKVRWLKKEMEKYADREDMIIMFVDSYDVILAGSPTELLKKFVQSGSRLLFSAESFCWPEWGLAEQYPEVGTGKRFLNSGGFIGFATTIHQIVRQWKYKDDDDDQLFYTRLYLDPGLREKLSLNLDHKSRIFQNLNGALDEVVLKFDRNRVRIRNVAYDTLPIVVHGNGPTKLQLNYLGNYVPNGWTPEGGCGFCNQDRRTLPGGQPPPRVFLAVFVEQPTPFLPRFLQRLLLLDYPPDRVTLFLHNNEVFHEPHIADSWPQLQDHFSAVKLVGPEEALSPGEARDMAMDLCRQDPECEFYFSLDADAVLTNLQTLRILIEENRKVIAPMLSRHGKLWSNFWGALSPDEYYARSEDYVELVQRKRVGVWNVPYISQAYVIRGDTLRMELPQRDVFSGSDTDPDMAFCKSFRDKGIFLHLSNQHEFGRLLATSRYDTEHLHPDLWQIFDNPVDWKEQYIHENYSRALEGEGIVEQPCPDVYWFPLLSEQMCDELVAEMEHYGQWSGGRHEDSRLAGGYENVPTVDIHMKQVGYEDQWLQLLRTYVGPMTESLFPGYHTKARAVMNFVVRYRPDEQPSLRPHHDSSTFTLNVALNHKGLDYEGGGCRFLRYDCVISSPRKGWALLHPGRLTHYHEGLPTTWGTRYIMVSFVDP

SEQ ID NO: 24 - protein, 45 aa, Artificial Sequence
  Vacuole signal sequence of barley gene for Thiol protease aleurain precursor
MAHARVLLLALAVLATAAVAVASSSSFADSNPIRPVTDRAASTLA

SEQ ID NO: 25 - DNA, 24 bp, Artificial Sequence
  Single strand DNA oligonucleotide
atcaccaggagaacagggaccatc

SEQ ID NO: 26 - DNA, 29 bp, Artificial Sequence
  Single strand DNA oligonucleotide
tccacttccaaatctctatccctaacaac

SEQ ID NO: 27 - DNA, 23 bp, Artificial Sequence
  Single strand DNA oligonucleotide
aggcattagaggcgataagggag

SEQ ID NO: 28 - DNA, 27 bp, Artificial Sequence
  Single strand DNA oligonucleotide
tcaatccaataatagccacttgaccac

SEQ ID NO: 29 - DNA, 102 bp, Artificial Sequence
  pBINPLUS multiple cloning site
atgaccatgattacgccaagctggcgcgccaagcttgcatgcctgcaggtcgactctagaggatccccgggtaccgagctcgaattcttaattaacaattca

SEQ ID NO: 30 - protein, 1464 aa, Homo sapiens
MFSFVDLRLLLLLAATALLTHGQEEGQVEGQDEDIPPITCVQNGLRYHDRDVWKPEPCRICVCDNGKVLCDDVICDETKNCPGAEVPEGECCPVCPDGSESPTDQETTGVEGPKGDTGPRGPRGPAGPPGRDGIPGQPGLPGPPGPPGPPGPPGLGGNFAPQLSYGYDEKSTGGISVPGPMGPSGPRGLPGPPGAPGPQGFQGPPGEPGEPGASGPMGPRGPPGPPGKNGDDGEAGKPGRPGERGPPGPQGARGLPGTAGLPGMKGHRGFSGLDGAKGDAGPAGPKGEPGSPGENGAPGQMGPRGLPGERGRPGAPGPAGARGNDGATGAAGPPGPTGPAGPPGFPGAVGAKGEAGPQGPRGSEGPQGVRGEPGPPGPAGAAGPAGNPGADGQPGAKGANGAPGIAGAPGFPGARGPSGPQGPGGPPGPKGNSGEPGAPGSKGDTGAKGEPGPVGVQGPPGPAGEEGKRGARGEPGPTGLPGPPGERGGPGSRGFPGADGVAGPKGPAGERGSPGPAGPKGSPGEAGRPGEAGLPGAKGLTGSPGSPGPDGKTGPPGPAGQDGRPGPPGPPGARGQAGVMGFPGPKGAAGEPGKAGERGVPGPPGAVGPAGKDGEAGAQGPPGPAGPAGERGEQGPAGSPGFQGLPGPAGPPGEAGKPGEQGVPGDLGAPGPSGARGERGFPGERGVQGPPGPAGPRGANGAPGNDGAKGDAGAPGAPGSQGAPGLQGMPGERGAAGLPGPKGDRGDAGPKGADGSPGKDGVRGLTGPIGPPGPAGAPGDKGESGPSGPAGPTGARGAPGDRGEPGPPGPAGFAGPPGADGQPGAKGEPGDAGAKGDAGPPGPAGPAGPPGPIGNVGAPGAKGARGSAGPPGATGFPGAAGRVGPPGPSGNAGPPGPPGPAGKEGGKGPRGETGPAGRPGEVGPPGPPGPAGEKGSPGADGPAGAPGTPGPQGIAGQRGVVGLPGQRGERGFPGLPGPSGEPGKQGPSGASGERGPPGPMGPPGLAGPPGESGREGAPGAEGSPGRDGSPGAKGDRGETGPAGPPGAPGAPGAPGPVGPAGKSGDRGETGPAGPAGPVGPVGARGPAGPQGPRGDKGETGEQGDRGIKGHRGFSGLQGPPGPPGSPGEQGPSGASGPAGPRGPPGSAGAPGKDGLNGLPGPIGPPGPRGRTGDAGPVGPPGPPGPPGPPGPPSAGFDFSFLPQPPQEKAHDGGRYYRADDANVVRDRDLEVDTTLKSLSQQIENIRSPEGSRKNPARTCRDLKMCHSDWKSGEYWIDPNQGCNLDAIKVFCNMETGETCVYPTQPSVAQKNWYISKNPKDKRHVWFGESMTDGFQFEYGGQGSDPADVAIQLTFLRLMSTEASQNITYHCKNSVAYMDQQTGNLKKALLLQGSNEIEIRAEGNSRFTYSVTVDGCTSHTGAWGKTVIEYKTTKTSRLPIIDVAPLDVGAPDQEFGFDVGPVCFL

SEQ ID NO: 31 - protein, 1366 aa, Homo sapiens [sequence omitted]

SEQ ID NO: 32 - DNA, 5927 bp, Homo sapiens
tcgtcggagcagacgggagtttctcctcggggtcggagcaggaggcacgcggagtgtgaggccacgcatgagcggacgctaaccccctccccagccacaaagagtctacatgtctagggtctagacatgttcagctttgtggacctccggctcctgctcctcttagcggccaccgccctcctgacgcacggccaagaggaaggccaagtcgagggccaagacgaagacatcccaccaatcacctgcgtacagaacggcctcaggtaccatgaccgagacgtgtggaaacccgagccctgccggatctgcgtctgcgacaacggcaaggtgttgtgcgatgacgtgatctgtgacgagaccaagaactgccccggcgccgaagtccccgagggcgagtgctgtcccgtctgccccgacggctcagagtcacccaccgaccaagaaaccaccggcgtcgagggacccaagggagacactggcccccgaggcccaaggggacccgcaggcccccctggccgagatggcatccctggacagcctggacttcccggaccccccggaccccccggacctcccggaccccctggcctcggaggaaactttgctccccagctgtcttatggctatgatgagaaatcaaccggaggaatttccgtgcctggccccatgggtccctctggtcctcgtggtctccctggcccccctggtgcacctggtccccaaggcttccaaggtccccctggtgagcctggcgagcctggagcttcaggtcccatgggtccccgaggtcccccaggtccccctggaaagaatggagatgatggggaagctggaaaacctggtcgtcctggtgagcgtgggcctcctgggcctcagggtgctcgaggattgcccggaacagctggcctccctggaatgaagggacacagaggtttcagtggtttggatggtgccaagggagatgctggtcctgctggtcctaagggtgagcctggcagccctggtgaaaatggagctcctggtcagatgggcccccgtggcctgcctggtgagagaggtcgccctggagcccctggccctgctggtgctcgtggaaatgatggtgctactggtgctgccgggccccctggtcccaccggccccgctggtcctcctggcttccctggtgctgttggtgctaagggtgaagctggtccccaagggccccgaggctctgaaggtccccagggtgtgcgtggtgagcctggcccccctggccctgctggtgctgctggccctgctggaaaccctggtgctgatggacagcctggtgctaaaggtgccaatggtgctcctggtattgctggtgctcctggcttccctggtgcccgaggcccctctggaccccagggccccggcggccctcctggtcccaagggtaacagcggtgaacctggtgctcctggcagcaaaggagacactggtgctaagggagagcctggccctgttggtgttcaaggaccccctggccctgctggagaggaaggaaagcgaggagctcgaggtgaacccggacccactggcctgcccggaccccctggcgagcgtggtggacctggtagccgtggtttccctggcgcagatggtgttgctggtcccaagggtcccgctggtgaacgtggttctcctggccctgctggccccaaaggatctcctggtgaagctggtcgtcccggtgaagctggtctgcctggtgccaagggtctgactggaagccctggcagccctggtcctgatggcaaaactggcccccctggtcccgccggtcaagatggtcgccccggacccccaggcccacctggtgcccgtggtcaggctggtgtgatgggattccctggacctaaaggtgctgctggagagcccggcaaggctggagagcgaggtgttcccggaccccctggcgctgtcggtcctgctggcaaagatggagaggctggagctcagggaccccctggccctgctggtcccgctggcgagagaggtgaacaaggccctgctggctcccccggattccagggtctccctggtcctgctggtcctccaggtgaagcaggcaaacctggtgaacagggtgttcctggagaccttggcgcccctggcccctctggagcaagaggcgagagaggtttccctggcgagcgtggtgtgcaaggtccccctggtcctgctggtccccgaggggccaacggtgctcccggcaacgatggtgctaagggtgatgctggtgcccctggagctcccggtagccagggcgcccctggccttcagggaatgcctggtgaacgtggtgcagctggtcttccagggcctaagggtgacagaggtgatgctggtcccaaaggtgctgatggctctcctggcaaagatggcgtccgtggtctgactggccccattggtcctcctggccctgctggtgcccctggtgacaagggtgaaagtggtcccagcggccctgctggtcccactggagctcgtggtgcccccggagaccgtggtgagcctggtccccccggccctgctggctttgctggcccccctggtgctgacggccaacctggtgctaaaggcgaacctggtgatgctggtgctaaaggcgatgctggtccccctggccctgccggacccgctggaccccctggccccattggtaatgttggtgctcctggagccaaaggtgctcgcggcagcgctggtccccctggtgctactggtttccctggtgctgctggccgagtcggtcctcctggcccctctggaaatgctggaccccctggccctcctggtcctgctggcaaagaaggcggcaaaggtccccgtggtgagactggccctgctggacgtcctggtgaagttggtccccctggtccccctggccctgctggcgagaaaggatcccctggtgctgatggtcctgctggtgctcctggtactcccgggcctcaaggtattgctggacagcgtggtgtggtcggcctgcctggtcagagaggagagagaggcttccctggtcttcctggcccctctggtgaacctggcaaacaaggtccctctggagcaagtggtgaacgtggtccccctggtcccatgggcccccctggattggctggaccccctggtgaatctggacgtgagggggctcctggtgccgaaggttcccctggacgagacggttctcctggcgccaagggtgaccgtggtgagaccggccccgctggaccccctggtgctcctggtgctcctggtgcccctggccccgttggccctgctggcaagagtggtgatcgtggtgagactggtcctgctggtcccgccggtcctgtcggccctgttggcgcccgtggccccgccggaccccaaggcccccgtggtgacaagggtgagacaggcgaacagggcgacagaggcataaagggtcaccgtggcttctctggcctccagggtccccctggccctcctggctctcctggtgaacaaggtccctctggagcctctggtcctgctggtccccgaggtccccctggctctgctggtgctcctggcaaagatggactcaacggtctccctggccccattgggccccctggtcctcgcggtcgcactggtgatgctggtcctgttggtccccccggccctcctggacctcctggtccccctggtcctcccagcgctggtttcgacttcagcttcctgccccagccacctcaagagaaggctcacgatggtggccgctactaccgggctgatgatgccaatgtggttcgtgaccgtgacctcgaggtggacaccaccctcaagagcctgagccagcagatcgagaacatccggagcccagagggcagccgcaagaaccccgcccgcacctgccgtgacctcaagatgtgccactctgactggaagagtggagagtactggattgaccccaaccaaggctgcaacctggatgccatcaaagtcttctgcaacatggagactggtgagacctgcgtgtaccccactcagcccagtgtggcccagaagaactggtacatcagcaagaaccccaaggacaagaggcatgtctggttcggcgagagcatgaccgatggattccagttcgagtatggcggccagggctccgaccctgccgatgtggccatccagctgaccttcctgcgcctgatgtccaccgaggcctcccagaacatcacctaccactgcaagaacagcgtggcctacatggaccagcagactggcaacctcaagaaggccctgctcctccagggctccaacgagatcgagatccgcgccgagggcaacagccgcttcacctacagcgtcactgtcgatggctgcacgagtcacaccggagcctggggcaagacagtgattgaatacaaaaccaccaagacctcccgcctgcccatcatcgatgtggcccccttggacgttggtgccccagaccaggaattcggcttcgacgttggccctgtctgcttcctgtaaactccctccatcccaacctggctccctcccacccaaccaactttccccccaacccggaaacagacaagcaacccaaactgaaccccctcaaaagccaaaaaatgggagacaatttcacatggactttggaaaatatttttttcctttgcattcatctctcaaacttagtttttatctttgaccaaccgaacatgaccaaaaaccaaaagtgcattcaaccttaccaaaaaaaaaaaaaaaaaaagaataaataaataactttttaaaaaaggaagcttggtccacttgcttgaagacccatgcgggggtaagtccctttctgcccgttgggcttatgaaaccccaatgctgccctttctgctcctttctccacaccccccttggggcctcccctccactccttcccaaatctgtctccccagaagacacaggaaacaatgtattgtctgcccagcaatcaaaggcaatgctcaaacacccaagtggcccccaccctcagcccgctcctgcccgcccagcacccccaggccctgggggacctggggttctcagactgccaaagaagccttgccatctggcgctcccatggctcttgcaacatctccccttcgtttttgagggggtcatgccgggggagccaccagcccctcactgggttcggaggagagtcaggaagggccacgacaaagcagaaacatcggatttggggaacgcgtgtcaatcccttgtgccgcagggctgggcgggagagactgttctgttccttgtgtaactgtgttgctgaaagactacctcgttcttgtcttgatgtgtcaccggggcaactgcctgggggcggggatgggggcagggtggaagcggctccccattttataccaaaggtgctacatctatgtgatgggtggggtggggagggaatcactggtgctatagaaattgagatgcccccccaggccagcaaatgttcctttttgttcaaagtctatttttattccttgatatttttctttttttttttttttttttgtggatggggacttgtgaatttttctaaaggtgctatttaacatgggaggagagcgtgtgcggctccagcccagcccgctgctcactttccaccctctctccacctgcctctggcttctcaggcctctgctctccgacctctctcctctgaaaccctcctccacagctgcagcccatcctcccggctccctcctagtctgtcctgcgtcctctgtccccgggtttcagagacaacttcccaaagcacaaagcagtttttccccctaggggtgggaggaagcaaaagactctgtacctattttgtatgtgtataataatttgagatgtttttaattattttgattgctggaataaagcatgtggaaatgacccaaacataa

SEQ ID NO: 33 - DNA, 5411 bp, Homo sapiens
gtgtcccatagtgtttccaaacttggaaagggcgggggagggcgggaggatgcggagggcggaggtatgcagacaacgagtcagagtttccccttgaaagcctcaaaagtgtccacgtcctcaaaaagaatggaaccaatttaagaagccagccccgtggccacgtcccttcccccattcgctccctcctctgcgcccccgcaggctcctcccagctgtggctgcccgggcccccagccccagccctcccattggtggaggcccttttggaggcaccctagggccagggaaacttttgccgtataaatagggcagatccgggctttattattttagcaccacggcagcaggaggtttcggctaagttggaggtactggccacgactgcatgcccgcgcccgccaggtgatacctccgccggtgacccaggggctctgcgacacaaggagtctgcatgtctaagtgctagacatgctcagctttgtggatacgcggactttgttgctgcttgcagtaaccttatgcctagcaacatgccaatctttacaagaggaaactgtaagaaagggcccagccggagatagaggaccacgtggagaaaggggtccaccaggccccccaggcagagatggtgaagatggtcccacaggccctcctggtccacctggtcctcctggcccccctggtctcggtgggaactttgctgctcagtatgatggaaaaggagttggacttggccctggaccaatgggcttaatgggacctagaggcccacctggtgcagctggagccccaggccctcaaggtttccaaggacctgctggtgagcctggtgaacctggtcaaactggtcctgcaggtgctcgtggtccagctggccctcctggcaaggctggtgaagatggtcaccctggaaaacccggacgacctggtgagagaggagttgttggaccacagggtgctcgtggtttccctggaactcctggacttcctggcttcaaaggcattaggggacacaatggtctggatggattgaagggacagcccggtgctcctggtgtgaagggtgaacctggtgcccctggtgaaaatggaactccaggtcaaacaggagcccgtgggcttcctggtgagagaggacgtgttggtgcccctggcccagctggtgcccgtggcagtgatggaagtgtgggtcccgtgggtcctgctggtcccattgggtctgctggccctccaggcttcccaggtgcccctggccccaagggtgaaattggagctgttggtaacgctggtcctgctggtcccgccggtccccgtggtgaagtgggtcttccaggcctctccggccccgttggacctcctggtaatcctggagcaaacggccttactggtgccaagggtgctgctggccttcccggcgttgctggggctcccggcctccctggaccccgcggtattcctggccctgttggtgctgccggtgctactggtgccagaggacttgttggtgagcctggtccagctggctccaaaggagagagcggtaacaagggtgagcccggctctgctgggccccaaggtcctcctggtcccagtggtgaagaaggaaagagaggccctaatggggaagctggatctgccggccctccaggacctcctgggctgagaggtagtcctggttctcgtggtcttcctggagctgatggcagagctggcgtcatgggccctcctggtagtcgtggtgcaagtggccctgctggagtccgaggacctaatggagatgctggtcgccctggggagcctggtctcatgggacccagaggtcttcctggttcccctggaaatatcggccccgctggaaaagaaggtcctgtcggcctccctggcatcgacggcaggcctggcccaattggcccagctggagcaagaggagagcctggcaacattggattccctggacccaaaggccccactggtgatcctggcaaaaacggtgataaaggtcatgctggtcttgctggtgctcggggtgctccaggtcctgatggaaacaatggtgctcagggacctcctggaccacagggtgttcaaggtggaaaaggtgaacagggtccccctggtcctccaggcttccagggtctgcctggcccctcaggtcccgctggtgaagttggcaaaccaggagaaaggggtctccatggtgagtttggtctccctggtcctgctggtccaagaggggaacgcggtcccccaggtgagagtggtgctgccggtcctactggtcctattggaagccgaggtccttctggacccccagggcctgatggaaacaagggtgaacctggtgtggttggtgctgtgggcactgctggtccatctggtcctagtggactcccaggagagaggggtgctgctggcatacctggaggcaagggagaaaagggtgaacctggtctcagaggtgaaattggtaaccctggcagagatggtgctcgtggtgctcctggtgctgtaggtgcccctggtcctgctggagccacaggtgaccggggcgaagctggggctgctggtcctgctggtcctgctggtcctcggggaagccctggtgaacgtggtgaggtcggtcctgctggccccaatggatttgctggtcctgctggtgctgctggtcaacctggtgctaaaggagaaagaggagccaaagggcctaagggtgaaaacggtgttgttggtcccacaggccccgttggagctgctggcccagctggtccaaatggtccccccggtcctgctggaagtcgtggtgatggaggcccccctggtatgactggtttccctggtgctgctggacggactggtcccccaggaccctctggtatttctggccctcctggtccccctggtcctgctgggaaagaagggcttcgtggtcctcgtggtgaccaaggtccagttggccgaactggagaagtaggtgcagttggtccccctggcttcgctggtgagaagggtccctctggagaggctggtactgctggacctcctggcactccaggtcctcagggtcttcttggtgctcctggtattctgggtctccctggctcgagaggtgaacgtggtctaccaggtgttgctggtgctgtgggtgaacctggtcctcttggcattgccggccctcctggggcccgtggtcctcctggtgctgtgggtagtcctggagtcaacggtgctcctggtgaagctggtcgtgatggcaaccctgggaacgatggtcccccaggtcgcgatggtcaacccggacacaagggagagcgcggttaccctggcaatattggtcccgttggtgctgcaggtgcacctggtcctcatggccccgtgggtcctgctggcaaacatggaaaccgtggtgaaactggtccttctggtcctgttggtcctgctggtgctgttggcccaagaggtcctagtggcccacaaggcattcgtggcgataagggagagcccggtgaaaaggggcccagaggtcttcctggcttaaagggacacaatggattgcaaggtctgcctggtatcgctggtcaccatggtgatcaaggtgctcctggctccgtgggtcctgctggtcctaggggccctgctggtccttctggccctgctggaaaagatggtcgcactggacatcctggtacagttggacctgctggcattcgaggccctcagggtcaccaaggccctgctggcccccctggtccccctggccctcctggacctccaggtgtaagcggtggtggttatgactttggttacgatggagacttctacagggctgaccagcctcgctcagcaccttctctcagacccaaggactatgaagttgatgctactctgaagtctctcaacaaccagattgagacccttcttactcctgaaggctctagaaagaacccagctcgcacatgccgtgacttgagactcagccacccagagtggagcagtggttactactggattgaccctaaccaaggatgcactatggatgctatcaaagtatactgtgatttctctactggcgaaacctgtatccgggcccaacctgaaaacatcccagccaagaactggtataggagctccaaggacaagaaacacgtctggctaggagaaactatcaatgctggcagccagtttgaatataatgtagaaggagtgacttccaaggaaatggctacccaacttgccttcatgcgcctgctggccaactatgcctctcagaacatcacctaccactgcaagaacagcattgcatacatggatgaggagactggcaacctgaaaaaggctgtcattctacagggctctaatgatgttgaacttgttgctgagggcaacagcaggttcacttacactgttcttgtagatggctgctctaaaaagacaaatgaatggggaaagacaatcattgaatacaaaacaaataagccatcacgcctgcccttccttgatattgcacctttggacatcggtggtgctgaccaggaattctttgtggacattggcccagtctgtttcaaataaatgaactcaatctaaattaaaaaagaaagaaatttgaaaaaactttctctttgccatttcttcttcttcttttttaactgaaagctgaatccttccatttcttctgcacatctacttgcttaaattgtgggcaaaagagaaaaagaaggattgatcagagcattgtgcaatacagtttcattaactccttcccccgctcccccaaaaatttgaatttttttttcaacactcttacacctgttatggaaaatgtcaacctttgtaagaaaaccaaaataaaaattgaaaaataaaaaccataaacatttgcaccacttgtggcttttgaatatcttccacagagggaagtttaaaacccaaacttccaaaggtttaaactacctcaaaacactttcccatgagtgtgatccacattgttaggtgctgacctagacagagatgaactgaggtccttgttttgttttgttcataatacaaaggtgctaattaatagtatttcagatacttgaagaatgttgatggtgctagaagaatttgagaagaaatactcctgtattgagttgtatcgtgtggtgtattttttaaaaaatttgatttagcattcatattttccatcttattcccaattaaaagtatgcagattatttgcccaaatcttcttcagattcagcatttgttctttgccagtctcattttcatcttcttccatggttccacagaagctttgtttcttgggcaagcagaaaaattaaattgtacctattttgtatatgtgagatgtttaaataaattgtgaaaaaaatgaaataaagcatgtttggttttccaaaagaacatat

SEQ ID NO: 34 - DNA, 1633 bp, Artificial Sequence; identical to SEQ ID NO: 12
  Synthetic sequence containing the coding regions of the vascular signal sequence of barley gene for Thiol protease aleurain precursor fused to the human Prolyl 4-hydroxylase beta subunit and flanking regions

SEQ ID NO: 35 - DNA, 1723 bp, Artificial Sequence; identical to SEQ ID NO: 14
  Synthetic sequence containing the coding regions of the vascular signal sequence of barley gene for Thiol protease aleurain precursor fused to the human Prolyl 4-hydroxylase alpha-1 subunit and flanking regions

SEQ ID NO: 36 - protein, 1489 aa, Homo sapiens; identical to SEQ ID NO: 3

SEQ ID NO: 37 - protein, 1389 aa, Homo sapiens; identical to SEQ ID NO: 6

SEQ ID NO: 38 - DNA, 2888 bp, Artificial Sequence; identical to SEQ ID NO: 22
  Synthetic sequence containing the coding regions of the vascular signal sequence of barley gene for Thiol protease aleurain precursor fused to the human Lysyl hydroxylase 3 and flanking regions

SEQ ID NO: 39 - DNA, 2689 bp, Artificial Sequence; identical to SEQ ID NO: 18
  Synthetic sequence containing the coding regions of the human Procollagen C-proteinase and flanking regions

SEQ ID NO: 40 - DNA, 2912 bp, Artificial Sequence; identical to SEQ ID NO: 20
  Synthetic sequence containing the coding regions of the human Procollagen I N-proteinase and flanking regions

SEQ ID NO: 41 - DNA, 4467 bp, Homo sapiens
atggctcacgctcgtgttctcctcctcgctctcgctgttttggcaacagctgctgtggctgtggcttctagttcttcttttgctgattcaaaccctattagacctgttactgatagagcagcttccactttggctcaattgcaagaggagggccaggttgagggccaagatgaggatatccctccaattacatgcgtgcaaaatggcttgcgttaccacgatagggatgtgtggaaacctgaaccttgtcgtatctgtgtgtgtgataacggcaaggtgctctgcgatgatgttatctgcgatgagacaaaaaattgccctggcgctgaagttcctgagggcgagtgttgccctgtgtgccctgatggttccgagtccccaactgatcaggaaactactggcgtggagggcccaaaaggagatactggtccacgtggtcctaggggtccagcaggtcctccaggtagagatggtattccaggccagcctggattgccaggaccaccaggcccacctggcccaccaggacctcctggtcttggtggaaatttcgctccacaactctcttatggctatgatgagaagtcaacaggtggtatttccgttccaggtcctatgggaccatccggaccaagaggtctcccaggtcctccaggtgctcctggacctcaaggctttcaaggacctccaggcgaaccaggagaaccaggcgcttctggaccaatgggcccaaggggaccacctggcccaccaggaaaaaatggcgatgatggcgaagctggaaagcctggtcgtcctggagagagaggtcctcctggcccacagggtgcaagaggcttgccaggaactgctggcttgcctggaatgaagggacataggggcttctccggcctcgatggcgctaagggtgatgctggccctgctggaccaaagggcgagccaggttcccctggagaaaacggtgctcctggacaaatgggtcctcgtggacttccaggagaaaggggtcgtccaggcgctccaggaccagcaggtgctaggggaaacgatggtgcaacaggcgctgctggccctcctggcccaactggtcctgctggccctccaggattcccaggcgcagttggagctaaaggagaagcaggaccacagggccctaggggttctgaaggacctcagggtgttagaggtgaaccaggtcctccaggcccagctggagcagctggtccagcaggaaatccaggtgctgatggtcaacctggagctaagggcgctaatggcgcaccaggtatcgcaggcgcaccaggttttcctggcgctagaggcccaagtggtcctcaaggaccaggtggaccaccaggtccaaaaggcaattctggcgaacctggcgctccaggttctaaaggagatactggtgctaaaggcgaaccaggacctgttggtgttcagggtcctcctggtcctgctggagaagaaggaaaaagaggtgctcgtggagaaccaggaccaactggacttcctggacctcctggtgaacgtggcggacctggctcaaggggtttccctggagctgatggagtggcaggtccaaaaggccctgctggagagagaggttcaccaggtccagctggtcctaagggctcccctggtgaagcaggtagaccaggcgaagcaggattgccaggcgcaaagggattgacaggctctcctggtagtcctggcccagatggaaaaacaggcccaccaggtccagcaggacaagatggacgtccaggcccaccaggtcctcctggagcaaggggacaagctggcgttatgggttttccaggacctaaaggtgctgctggagagccaggaaaggcaggtgaaagaggagttcctggtccaccaggagcagtgggtcctgctggcaaagatggtgaagctggagcacagggccctccaggccctgctggcccagctggcgaacgtggagaacaaggcccagctggtagtccaggatttcaaggattgcctggccctgctggccctccaggagaagcaggaaaacctggagaacaaggagttcctggtgatttgggagcacctggaccttcaggagcacgtggtgaaagaggcttccctggcgagaggggtgttcaaggtccaccaggtccagcaggacctagaggtgctaatggcgctcctggcaacgatggagcaaaaggtgatgctggtgctcctggcgcacctggaagtcagggtgctcctggattgcaaggaatgcctggagagaggggtgctgctggcttgccaggcccaaagggcgataggggtgatgctggaccaaaaggtgctgatggatccccaggaaaagatggagttcgtggtcttactggcccaatcggacctccaggccctgctggcgctccaggtgataagggcgaaagtggcccaagtggacctgctggacctactggtgctagaggtgcacctggtgataggggtgaacctggaccacctggtccagctggttttgctggtcctcctggagctgatggacaacctggcgcaaagggtgaaccaggtgatgctggcgcaaagggagatgctggtccacctggacctgctggtccagcaggcccccctgggccaatcggtaatgttggagcaccaggtgctaagggagctaggggttccgctggtccacctggagcaacaggatttccaggcgctgctggtagagttggcccaccaggcccatccggaaacgcaggccctcctggtcctccaggtcctgctggcaaggagggtggcaaaggaccaaggggcgaaactggccctgctggtagacctggcgaagttggccctcctggaccaccaggtccagcaggagaaaaaggttccccaggagctgatggcccagctggtgctccaggaactccaggccctcaaggtattgctggacagagaggcgttgtgggactccctggtcaaaggggagagagaggatttccaggcttgccaggacctagtggagaacctggaaaacaaggcccatcaggcgctagtggagagcgtggacctcctggccctatgggacctcctggattggctggcccacctggcgaatcaggtcgtgaaggcgcaccaggcgcagaaggatcacctggaagagatggatcccctggtgctaaaggcgatcgtggagaaactggtccagcaggcccaccaggcgcaccaggtgcacctggcgctccaggacctgtgggaccagctggaaaatccggagataggggcgagacaggcccagcaggaccagctggacctgttggccctgctggcgctcgtggaccagcaggacctcaaggaccaaggggagataagggagaaacaggcgaacaaggcgataggggcattaagggtcataggggttttagtggcctccagggtcctcctggcccacctggatcaccaggagaacagggaccatctggtgcttccggcccagctggtccaagaggacctccaggatcagctggtgcacctggaaaagatggtcttaacggtctcccaggaccaatcggccctccaggacctagaggaagaacaggagatgctggccctgttggccctccaggacctcctggtccaccaggtccacctggtcctccatcagctggattcgatttttcatttcttccacagccaccacaagagaaagctcacgatggcggcagatattaccgtgctgatgatgctaacgttgttagggatagagatttggaagtggatacaactttgaaatccctctcccagcaaattgaaaacattagatctccagaaggttcacgtaaaaacccagctagaacatgtcgtgatttgaaaatgtgtcactccgattggaaaagtggtgaatactggattgatccaaatcagggctgtaatctcgatgctatcaaagttttctgtaacatggaaacaggcgaaacatgcgtttatcctactcaaccttccgtggctcagaaaaattggtacatctcaaaaaatcctaaagataagaggcacgtttggttcggtgaaagtatgactgatggatttcaatttgagtacggcggtcaaggtagtgatccagctgatgtggctattcaactcacatttttgcgtcttatgtccacagaggcatcacaaaacatcacttaccactgcaaaaacagtgtggcttatatggatcaacaaacaggaaaccttaagaaggctcttcttttgaagggctcaaacgagattgagattagagcagagggcaactcaaggtttacttattcagttactgttgatggctgcacttcacatactggcgcttggggtaaaacagttatcgagtataagactacaaaaacatcaagactcccaatcattgatgttgctcctctcgatgttggcgctcctgatcaagagttcggttttgatgtgggcccagtttgtttcctc

SEQ ID NO: 42 - DNA, 4167 bp, Homo sapiens
atggctcacgctcgtgttctcctcctcgctctcgctgttttggcaacagctgctgtggctgtggcttcaagttctagttttgctgattccaacccaattcgtccagttactgatagagcagcttccactttggctcaattgcttcaagaagaaactgtgaggaagggccctgctggcgataggggccctaggggcgaaaggggtccaccaggacctccaggcagggatggcgaagatggtccaactggccctcctggacctcctggccctccagggccacccggcttgggcggaaacttcgcagctcaatacgatggcaagggtgttggtcttggtcctggtcctatgggcttgatgggacctagaggcccacctggtgctgctggtgctcctggaccacagggttttcagggaccagctggcgagccaggagagccaggccaaacaggaccagctggtgcaaggggacctgctggacctcctggaaaagctggtgaagatggtcacccaggcaaaccaggacgtcctggcgaaagaggtgttgttggaccacaaggcgctaggggatttccaggtacacctggattgccaggttttaagggcattcgtggtcataacggcctcgatggattgaagggacagcctggcgcacctggcgttaagggtgaacctggagcaccaggtgaaaacggtactcctggccagactggtgcaagaggactcccaggtgaaaggggtagagttggtgctcctggacctgctggagctaggggtagtgatggtagtgttggtcctgtgggccctgctggtccaatcggttccgctggcccacctggattcccaggcgctccaggacctaaaggagaaatcggtgctgtgggtaacgcaggtcctactggtccagcaggtcctcgtggagaagtgggattgccaggactttctggtccagtgggccctccaggcaaccctggagctaacggcttgacaggagctaaaggcgcagcaggactccctggagtggctggcgcaccaggattgcctggtccaaggggtatcccaggccctgttggcgcagctggagctactggtgcacgtggacttgttggcgaaccaggccctgctggatcaaaaggcgagtctggaaataagggagaacctggttctgctggacctcaaggtcctcctggaccttctggagaagaaggaaaaaggggaccaaatggcgaggctggatcagcaggtccaccaggaccacctggacttcgtggatcccctggtagtagaggacttccaggcgctgatggtagagcaggcgttatgggaccaccaggaagtagaggagcatccggtccagcaggagttaggggtcctaacggagatgctggtagaccaggtgaaccaggtcttatgggcccaaggggcctcccaggtagtccaggaaatatcggccctgctggaaaagaaggccctgttggacttccaggtattgatggacgtcctggccctattggcccagcaggtgcaagaggagaacctggcaatattggatttccaggaccaaagggtccaacaggcgatcctggaaaaaatggagataagggtcatgctggattggcaggcgcaaggggcgctcctggtccagatggaaacaacggcgcacagggtccacctggccctcagggtgttcaaggcggaaaaggcgaacaaggcccagctggaccaccaggctttcaaggcttgccaggaccaagtggtccagcaggtgaagttggcaagccaggcgagcgtggacttcatggcgagtttggactccctggaccagcaggaccaaggggtgaaagaggccctcctggagagagtggcgctgctggaccaacaggcccaatcggtagtagaggtcctagtggacctccaggcccagatggaaataagggtgaaccaggagttgtgggcgctgttggaacagctggtccttcaggaccatcaggactcccaggcgagagaggcgctgctggcattcctggaggaaaaggtgaaaaaggcgaacctggcctccgtggcgaaatcggaaatcctggacgtgatggtgctcgtggtgcacacggcgctgtgggcgctccaggccctgctggtgctactggtgatagaggagaggctggcgcagctggcccagcaggtcctgctggcccaaggggtagtcctggtgaaagaggcgaagttggacctgctggccctaacggctttgctggccctgctggagcagcaggtcaacctggcgctaaaggtgaaaggggcggaaagggcccaaaaggtgaaaatggcgttgtgggaccaactggtccagtgggcgcagctggacctgctggtccaaatggaccaccaggaccagcaggtagtagaggagatggtggacctccaggaatgacaggttttccaggtgctgctggtagaacaggacctcctggtcctagtggtatttctggtccaccaggaccaccaggtcctgctggaaaagaaggattgaggggtccacgtggtgatcaaggaccagtgggcagaactggtgaagttggcgcagtgggaccacctggttttgctggagaaaagggcccttctggagaggcaggaacagctggtcctcctggtacacctggacctcaaggacttttgggtgcacctggtattctcggattgccaggaagtaggggcgaacgtggacttcctggcgtggcaggagcagttggagaacctggccctctcggaatcgcaggcccaccaggcgcaagaggaccaccaggagctgttggatcaccaggcgtgaatggtgcacctggcgaggctggtcgtgatggaaacccaggaaatgatggcccaccaggaagagatggtcaacctggacacaaaggcgagaggggctacccaggaaatattggcccagttggtgctgctggcgcaccaggcccacacggtccagttggaccagcaggaaaacacggtaatcgtggcgaaacaggcccttcaggcccagtgggacctgctggtgctgttggcccaagaggaccatctggacctcaaggcattagaggcgataagggagagcctggcgaaaaaggacctagaggcttgcctggttttaaaggacacaacggtctccaaggacttccaggtatcgctggtcatcatggagatcagggtgctcctggatcagtgggtccagcaggtcctagaggcccagcaggcccttccggtccagcaggaaaggatggacgtactggccaccctggaactgtgggccctgctggaattagaggtcctcaaggtcatcagggccctgctggccctccaggtccaccaggtcctccaggcccaccaggagtttcaggtggtggttacgattttggttacgatggtgatttttaccgtgctgatcaacctagaagtgctccttctctccgtcctaaagattatgaagttgatgctactttgaaatcacttaacaaccagattgagactcttctcacacctgagggatcaagaaagaatccagcacgtacatgccgtgatctcagacttagtcacccagagtggtcaagtggctattattggattgatcctaatcagggttgtacaatggaggctatcaaagtttactgtgattttccaactggagagacatgtattagggcacaacctgagaacattccagctaaaaattggtatcgttcctctaaagataagaaacatgtttggctcggagagactattaacgctggttctcagttcgagtataatgttgagggcgttacttctaaagagatggcaactcagctcgcttttatgagattgctcgctaactacgcatcccaaaacatcacttatcactgcaaaaattccattgcatatatggatgaggagacaggaaatttgaagaaagcagttattctccaaggtagtaacgatgttgagcttgtggctgagggaaatagtagattcacttacacagttttggtggatggatgctcaaagaaaactaatgagtggggcaagacaatcattgagtacaagacaaataagccttctaggctcccatttctcgatattgcacctcttgatatcggaggagctgatcacgagttttttgttgatatcggacctgtttgttttaag